European Patent Application EP 4 803 096 A1, published September 9, 2026. Title: Composition for prevention or treatment of bladder cancer. Applicant: GENOMICTREE, INC. The sequence listing filed with the application follows.

SEQUENCE LISTING (13 sequences)

SEQ ID NO: 1 - DNA, 804 bp, synthetic construct
  misc_feature 1..804: note = Synthetic Sequence
  source 1..804: mol_type = other DNA
atggcgcggttcctgacactttgcacttggctgctgttgctcggccccgggctcctggcgaccgtgcgggccgaatgcagccaggattgcgcgacgtgcagctaccgcctagtgcgcccggccgacatcaacttcctggcttgcgtaatggaatgtgaaggtaaactgccttctctgaaaatttgggaaacctgcaaggagctcctgcagctgtccaaaccagagcttcctcaagatggcaccagcaccctcagagaaaatagcaaaccggaagaaagccatttgctagccaaaaggtatgggggcttcatgaaaaggtatggaggcttcatgaagaaaatggatgagctttatcccatggagccagaagaagaggccaatggaagtgagatcctcgccaagcggtatgggggcttcatgaagaaggatgcagaggaggacgactcgctggccaattcctcagacctgctaaaagagcttctggaaacaggggacaaccgagagcgtagccaccaccaggatggcagtgataatgaggaagaagtgagcaagagatatgggggcttcatgagaggcttaaagagaagcccccaactggaagatgaagccaaagagctgcagaagcgatatgggggcttcatgagaagagtaggtcgcccagagtggtggatggactaccagaaacggtatggaggtttcctgaagcgctttgccgaggctctgccctccgacgaagaaggcgaaagttactccaaagaagttcctgaaatggaaaaaagatacggaggatttatgagattttaa

SEQ ID NO: 2 - DNA, 83 bp, synthetic construct
  misc_feature 1..83: note = Synthetic Sequence
  source 1..83: mol_type = other DNA
attaaaggtttataccttcccaggtaacaaaccaaccaactttcgatctcttgtagatctgttctctaaacgaacaaactaaa

SEQ ID NO: 3 - DNA, 196 bp, synthetic construct
  misc_feature 1..196: note = Synthetic Sequence
  source 1..196: mol_type = other DNA
caatctttaatcagtgtgtaacattagggaggacttgaaagagccaccacattttcaccgaggccacgcggagtacgatcgagtgtacagtgaacaatgctagggagagctgcctatatggaagagccctaatgtgtaaaattaattttagtagtgctatccccatgtgattttaatagcttcttaggagaatgac

SEQ ID NO: 4 - DNA, 1173 bp, synthetic construct
  misc_feature 1..1173: note = Synthetic Sequence
  source 1..1173: mol_type = other DNA
taatacgactcactatagggattaaaggtttataccttcccaggtaacaaaccaaccaactttcgatctcttgtagatctgttctctaaacgaacaaactaaaatggcgcggttcctgacactttgcacttggctgctgttgctcggccccgggctcctggcgaccgtgcgggccgaatgcagccaggattgcgcgacgtgcagctaccgcctagtgcgcccggccgacatcaacttcctggcttgcgtaatggaatgtgaaggtaaactgccttctctgaaaatttgggaaacctgcaaggagctcctgcagctgtccaaaccagagcttcctcaagatggcaccagcaccctcagagaaaatagcaaaccggaagaaagccatttgctagccaaaaggtatgggggcttcatgaaaaggtatggaggcttcatgaagaaaatggatgagctttatcccatggagccagaagaagaggccaatggaagtgagatcctcgccaagcggtatgggggcttcatgaagaaggatgcagaggaggacgactcgctggccaattcctcagacctgctaaaagagcttctggaaacaggggacaaccgagagcgtagccaccaccaggatggcagtgataatgaggaagaagtgagcaagagatatgggggcttcatgagaggcttaaagagaagcccccaactggaagatgaagccaaagagctgcagaagcgatatgggggcttcatgagaagagtaggtcgcccagagtggtggatggactaccagaaacggtatggaggtttcctgaagcgctttgccgaggctctgccctccgacgaagaaggcgaaagttactccaaagaagttcctgaaatggaaaaaagatacggaggatttatgagattttaacaatctttaatcagtgtgtaacattagggaggacttgaaagagccaccacattttcaccgaggccacgcggagtacgatcgagtgtacagtgaacaatgctagggagagctgcctatatggaagagccctaatgtgtaaaattaattttagtagtgctatccccatgtgattttaatagcttcttaggagaatgacaaaaaaaaaaaaaaaaaaaaaaaaaaaaaaaaaaaaaaaaaaaaaaaaaaaaaaaaaaaaaaaaatgcat

SEQ ID NO: 5 - DNA, 44 bp, synthetic construct
  misc_feature 1..44: note = Synthetic Sequence
  source 1..44: mol_type = other DNA
taatacgactcactatagggattaaaggtttataccttcccagg

SEQ ID NO: 6 - DNA, 28 bp, synthetic construct
  misc_feature 1..28: note = Synthetic Sequence
  source 1..28: mol_type = other DNA
tttagtttgttcgtttagagaacagatc

SEQ ID NO: 7 - DNA, 40 bp, synthetic construct
  misc_feature 1..40: note = Synthetic Sequence
  source 1..40: mol_type = other DNA
ctctaaacgaacaaactaaacaatctttaatcagtgtgta

SEQ ID NO: 8 - DNA, 89 bp, synthetic construct
  misc_feature 1..89: note = Synthetic Sequence
  source 1..89: mol_type = other DNA
tttttttttttttttttttttttttttttttttttttttttttttttttttttttttttttttttgtcattctcctaagaagctattaa

SEQ ID NO: 9 - DNA, 28 bp, synthetic construct
  misc_feature 1..28: note = Synthetic Sequence
  source 1..28: mol_type = other DNA
caatctttaatcagtgtgtaacattagg

SEQ ID NO: 10 - DNA, 39 bp, synthetic construct
  misc_feature 1..39: note = Synthetic Sequence
  source 1..39: mol_type = other DNA
ctctaaacgaacaaactaaaatggcgcggttcctgacac

SEQ ID NO: 11 - DNA, 46 bp, synthetic construct
  misc_feature 1..46: note = Synthetic Sequence
  source 1..46: mol_type = other DNA
tacacactgattaaagattgttaaaatctcataaatcctccgtatc

SEQ ID NO: 12 - DNA, 20 bp, synthetic construct
  misc_feature 1..20: note = Synthetic Sequence
  source 1..20: mol_type = other DNA
tccactagtaacggccgcca

SEQ ID NO: 13 - RNA, 1251 nt, synthetic construct
  misc_feature 1..1251: note = Synthetic Sequence
  source 1..1251: mol_type = other RNA
gggacggcgaggcaggcgctcagagccccgcagcctggcccgtgaccccgcagagacgctgaggaccgcgacgagtcgtgtctgaacccggcttttccaattggcctgctccatccgaacagcgtcaactccatggcgcggttcctgacactttgcacttggctgctgttgctcggccccgggctcctggcgaccgtgcgggccgaatgcagccaggattgcgcgacgtgcagctaccgcctagtgcgcccggccgacatcaacttcctggcttgcgtaatggaatgtgaaggtaaactgccttctctgaaaatttgggaaacctgcaaggagctcctgcagctgtccaaaccagagcttcctcaagatggcaccagcaccctcagagaaaatagcaaaccggaagaaagccatttgctagccaaaaggtatgggggcttcatgaaaaggtatggaggcttcatgaagaaaatggatgagctttatcccatggagccagaagaagaggccaatggaagtgagatcctcgccaagcggtatgggggcttcatgaagaaggatgcagaggaggacgactcgctggccaattcctcagacctgctaaaagagcttctggaaacaggggacaaccgagagcgtagccaccaccaggatggcagtgataatgaggaagaagtgagcaagagatatgggggcttcatgagaggcttaaagagaagcccccaactggaagatgaagccaaagagctgcagaagcgatatgggggcttcatgagaagagtaggtcgcccagagtggtggatggactaccagaaacggtatggaggtttcctgaagcgctttgccgaggctctgccctccgacgaagaaggcgaaagttactccaaagaagttcctgaaatggaaaaaagatacggaggatttatgagattttaatatcttttcccactagtggccccaggccccagcaagcctccctccatcctccagtgggaaactgttgatggtgttttattgtcatgtgttgcttgccttgtatagttgacttcattgtctggataactatacaacctgaaaactgtcatttcaggttctgtgctctttttggagtctttaagctcagtattagtctattgcagctatctcgttttcatgctaaaatagtttttgttatcttgtctcttatttttgacaaacatcaataaatgcttacttgtatatagagataataaacctattaccccaagtgca